European Patent Application EP 4 480 490 A1, published December 25, 2024. Title: BRICK1 for use in treating myocardial diseases. Applicant: Medizinische Hochschule Hannover. Application EP. The sequence listing filed with the application follows.

SEQUENCE LISTING (4 sequences)

SEQ ID NO: 1 - protein, 75 aa, Homo sapiens
MAGQEDPVQREIHQDWANREYIEIITSSIKKIADFLNSFDMSCRSRLATLNEKLTALERRIEYIEARVTKGETLT

SEQ ID NO: 2 - protein, 75 aa, Mus musculus
MAGQEDPVQREIHQDWANREYIEIITSSIKKISDFLNSFDMSCRSRLATLNEKLTALERRIEYIEARVTKGETLT

SEQ ID NO: 3 - DNA, 228 bp, Homo sapiens
  source 1..228: mol_type = other DNA
atggcgggacaggaggatccggtgcagcgggagattcaccaggactgggctaaccgggagtacattgagataatcaccagcagcatcaagaaaatcgcagactttctcaactcgttcgatatgtcttgtcgttcaagacttgcaacactaaacgagaaattgacagcccttgaacggagaatagagtacattgaagctcgggtgacaaaaggtgagacactcacctag

SEQ ID NO: 4 - DNA, 228 bp, Mus musculus
  source 1..228: mol_type = other DNA
atggcgggacaagaggatccggtgcagcgggagattcaccaggactgggcgaaccgggagtacattgagatcatcaccagcagcatcaagaaaatctcagactttctcaactctttcgatatgtcttgtcgttcaagactcgcaacactaaatgagaaattgacagcccttgaacggagaatagagtacattgaagcgagggtgacaaagggtgagactctgacctag